European Patent Specification EP 3 375 873 B1, published July 2, 2025. Title: Immunoglobulin binding peptide. Applicant: ProteNova Co., Ltd. The sequence listing filed with the application follows.

SEQUENCE LISTING (39 sequences)

SEQ ID NO: 1 - protein, 70 aa, Peptostreptococcus magnus
ETPEEPKEEVTIKVNLIFADGKTQTAEFKGTFEEATAEAYRYADLLAKVNGEYTADLEDGGYTINIKFAG

SEQ ID NO: 2 - protein, 70 aa, Peptostreptococcus magnus
ETPEEPKEEVTIKVNLIFADGKIQTAEFKGTFEEATAKAYAYANLLAKENGEYTADLEDGGNTINIKFAG

SEQ ID NO: 3 - protein, 70 aa, Peptostreptococcus magnus
EKPEEPKEEVTIKVNLIFADGKTQTAEFKGTFEEATAKAYAYADLLAKENGEYTADLEDGGNTINIKFAG

SEQ ID NO: 4 - protein, 69 aa, Peptostreptococcus magnus
ETPEPEEEVTIKANLIFADGSTQNAEFKGTFAKAVSDAYAYADALKKDNGEYTVDVADKGLTLNIKFAG

SEQ ID NO: 5 - protein, 992 aa, Peptostreptococcus magnus
MKINKKLLMAALAGAIVVGGGANAYAAEEDNTDNNLSMDEISDAYFDYHGDVSDSVDPVEEEIDEALAKALAEAKETAKKHIDSLNHLSETAKKLAKNDIDSATTINAINDIVARADVMERKTAEKEEAEKLAAAKETAKKHIDELKHLADKTKELAKRDIDSATTINAINDIVARADVMERKTAEKEEAEKLAAAKETAKKHIDELKHLADKTKELAKRDIDSATTIDAINDIVARADVMERKLSEKETPEPEEEVTIKANLIFADGSTQNAEFKGTFAKAVSDAYAYADALKKDNGEYTVDVADKGLTLNIKFAGKKEKPEEPKEEVTIKVNLIFADGKTQTAEFKGTFEEATAKAYAYADLLAKENGEYTADLEDGGNTINIKFAGKETPETPEEPKEEVTIKVNLIFADGKIQTAEFKGTFEEATAKAYAYANLLAKENGEYTADLEDGGNTINIKFAGKETPETPEEPKEEVTIKVNLIFADGKTQTAEFKGTFEEATAEAYRYADLLAKVNGEYTADLEDGGYTINIKFAGKEQPGENPGITIDEWLLKNAKEEAIKELKEAGITSDLYFSLINKAKTVEGVEALKNEILKAHAGEETPELKDGYATYEEAEAAAKEALKNDDVNNAYEIVQGADGRYYYVLKIEVADEEEPGEDTPEVQEGYATYEEAEAAAKEALKEDKVNNAYEVVQGADGRYYYVLKIEDKEDEQPGEEPGENPGITIDEWLLKNAKEDAIKELKEAGISSDIYFDAINKAKTVEGVEALKNEILKAHAEKPGENPGITIDEWLLKNAKEAAIKELKEAGITAEYLFNLINKAKTVEGVESLKNEILKAHAEKPGENPGITIDEWLLKNAKEDAIKELKEAGITSDIYFDAINKAKTIEGVEALKNEILKAHKKDEEPGKKPGEDKKPEDKKPGEDKKPEDKKPGEDKKPEDKKPGKTDKDSPNKKKKAKLPKAGSEAEILTLAAAALSTAAGAYVSLKKRK

SEQ ID NO: 6 - DNA, 3258 bp, Peptostreptococcus magnus
tttggacagtggacgaaacaagaacactgatttaataaattggtgaaattcgattgttgaaatacctttttgggtagaaataactaaggaatggcaatataattgcttggaaacgaatttgatttaaatagcattaaatgcaaaaaatttaaaaggaggagacaaattccaccctttataaagggaagtttccattgtcaaaataatatgaagattaataagaaattattaatggctgcacttgcaggagcaattgtagttggtggtggagctaacgcttacgcagctgaagaagataacactgataataacctttcaatggatgaaattagtgatgcttattttgattatcacggagatgtttcagattcagtagatcctgtagaagaagaaatagacgaagcattagcaaaagcattagcagaagctaaagaaacagcaaaaaaacatatagattctttaaatcatttgtcagaaacagcaaaaaaattagctaagaatgatatagattcagctactactattaatgcaatcaatgacatcgtagcaagagcagatgtaatggaaagaaaaacagctgaaaaagaagaagcagaaaaattagcagcagcaaaagaaacagcaaagaaacatatagatgaattaaaacacttagcagacaaaacaaaagaattagctaagagagatatagattcagctactactattaatgcaatcaatgacatcgtagcaagagcagatgtaatggaaagaaaaacagctgaaaaagaagaagcagaaaaattagcagcagcaaaagaaacagcaaagaaacatatagatgaattaaaacacttagcagacaaaacaaaagaattagctaagagagatatagattcagctactactattgatgcaatcaatgatatcgtagctagagcagatgtaatggaaagaaagttatctgaaaaagaaacaccagaaccagaagaagaagttacaatcaaagctaacttaatctttgcagatggaagcacacaaaatgcagaattcaaaggaacattcgcaaaagcagtatcagatgcttacgcttacgcagatgctttaaagaaagacaacggagaatatactgtagacgttgcagataaaggcttaactttaaatattaaattcgctggtaaaaaagaaaaaccagaagaaccaaaagaagaagttacaatcaaagttaacttaatctttgcagatggaaagacacaaacagcagaattcaaaggaacatttgaagaagcaacagcaaaagcttatgcttatgcagacttattagcaaaagaaaatggcgaatatacagcagacttagaagatggtggaaacacaatcaacattaaatttgctggaaaagaaacaccagaaacaccagaagaaccaaaagaagaagttacaatcaaagttaacttaatctttgcagatggaaagatacaaacagcagaattcaaaggaacatttgaagaagcaacagcaaaagcttatgcttatgcaaacttattagcaaaagaaaatggcgaatatacagcagacttagaagatggtggaaacacaatcaacattaaatttgctggaaaagaaacaccagaaacaccagaagaaccaaaagaagaagttacaatcaaagttaacttaatctttgcagatggaaaaacacaaacagcagaattcaaaggaacatttgaagaagcaacagcagaagcttacagatatgcagacttattagcaaaagtaaatggtgaatacacagcagacttagaagatggcggatacactatcaacatcaaatttgctggaaaagaacaaccaggcgaaaatccaggaatcacaattgatgaatggttattaaagaatgctaaagaagaagcaatcaaagaattaaaagaagcaggaatcacttctgatttatacttcagcttaatcaataaagcaaaaacagttgaaggcgtagaagcattaaagaacgaaatcttaaaagcacacgctggagaagaaacaccagaattaaaagatggatatgcaacatatgaagaagcagaagcagcagctaaagaagctttgaaaaatgatgatgttaacaacgcatacgaaatagttcaaggtgcagacggaagatactactatgtattaaagattgaagttgcagacgaagaagaaccaggtgaagacactccagaagttcaagaaggttacgcaacttacgaagaagcagaagcagcagctaaagaagcattaaaagaagataaagttaacaatgcatacgaagtagttcaaggtgcagacggaagatactactatgtattaaaaatcgaagataaagaagatgaacaaccaggtgaagaaccaggcgaaaacccaggaatcacaattgatgaatggttattaaagaatgctaaagaagacgcaatcaaagaattaaaagaagcaggaatcagttctgacatatactttgatgcaatcaacaaagcaaaaacagtagaaggcgtagaagcgttaaagaacgaaatcttaaaagcacacgctgaaaaaccaggcgaaaacccaggaatcacaattgatgaatggttattaaagaatgctaaagaagctgcaatcaaagaattaaaagaagcaggaatcactgctgaatatctattcaacttaatcaacaaagcaaaaacagtagaaggcgtagaatcattaaagaacgaaatcttaaaagcacacgctgaaaaaccaggcgaaaacccaggaatcacaattgatgaatggttattaaagaacgctaaagaagatgcaattaaagaattaaaagaagcaggaattacttctgacatatactttgatgctatcaacaaagcaaaaactattgaaggcgtagaagcattaaagaatgaaatcttaaaggctcataaaaaagatgaagaaccaggtaaaaaaccaggtgaagacaaaaaaccagaagataaaaaaccaggtgaagataaaaaaccagaagacaaaaaacctggtgaagataaaaaaccagaagacaaaaaaccaggtaaaacagataaagattctccaaataagaagaaaaaagctaaattaccaaaagctggtagcgaagctgaaatcttaacattagcagcagcagctttatcaacagcagcaggtgcttacgtttcacttaaaaaacgtaaataattaatcttagataaagaatagattaatataaaaaatgggacttataatagtcccattttttaatgcgaaaaa

SEQ ID NO: 7 - DNA, 210 bp, Artificial Sequence
  Modified DNA fragment of immunoglobulin kappa light chain binding domain 4 of protein L
gagaccccggaagaaccgcgcgaggaagtgacgatccgcgttaacctgatctttgcggatgggcgcacccagacggctgaattccgtggcaccttcgaagaggcgaccgcggaggcctaccgctatgcagatctcctcgccaaggtgaacggggaatatacggccgatcttgaggatggcgggtatacgatcaacattaaatttgcgggg

SEQ ID NO: 8 - DNA, 60 bp, Artificial Sequence
  oligo-166
ctggcggggctcgcattagagaagccggaagaaccgaaggaggaagtgacgatcaaggtt

SEQ ID NO: 9 - DNA, 58 bp, Artificial Sequence
  oligo-167
tgaattcagccgtctgggtcttcccatccgcaaagatcaggttaaccttgatcgtcac

SEQ ID NO: 10 - DNA, 67 bp, Artificial Sequence
  oligo-168
tgaattcaaaggcaccttcgaagaggcgaccgcggaggcctaccgctatgcagatctcctcgccaag

SEQ ID NO: 11 - DNA, 67 bp, Artificial Sequence
  oligo-169
tgttgatcgtatacccgccatcctcaagatcggccgtatattccccgttcaccttggcgaggagatc

SEQ ID NO: 12 - protein, 11 aa, Artificial Sequence
  Artifical sequence of N-terminal
MAQHDEAGLAL

SEQ ID NO: 13 - DNA, 50 bp, Artificial Sequence
  oligo-178
acaggcgctagcatatggcacagcatgacgaggcggggctcgcattagag

SEQ ID NO: 14 - DNA, 60 bp, Artificial Sequence
  oligo-170
gcggatcctattattagcgcggcgctaaggcccccgcaaatttaatgttgatcgtatacc

SEQ ID NO: 15 - DNA, 43 bp, Artificial Sequence
  oligo-189
tttgcgggggccttaccgagcaagagcaaaaaaatcttaaagg

SEQ ID NO: 16 - DNA, 37 bp, Artificial Sequence
  oligo-191
gcggatcctattatttcttctttttcggagcctgggc

SEQ ID NO: 17 - protein, 21 aa, Artificial Sequence
  Modified third alpha helix of immunoglobulin binding C domain of protein A
PSKSKKILKEAKKLNKAQAPK

SEQ ID NO: 18 - protein, 3 aa, Artificial Sequence
  Artificial sequence of C-terminal
KKK

SEQ ID NO: 19 - DNA, 69 bp, Artificial Sequence
  oligo-193
ggctcgcattagagacgccggaaccggaggaagaggtgacgatcaaggctaacctgatctttgcggatg

SEQ ID NO: 20 - DNA, 67 bp, Artificial Sequence
  oligo-194
catcgctcaccgcctttgcgaaggtgcctttgaattcagcgttctgggtgctcccatccgcaaagat

SEQ ID NO: 21 - DNA, 69 bp, Artificial Sequence
  oligo-195
cggtgagcgatgcctacgcgtatgcagatgcgctgaaaaaggacaacggggaatatacggtagacgtgg

SEQ ID NO: 22 - DNA, 66 bp, Artificial Sequence
  oligo-196
gctcggtaaggcccccgcaaatttaatgttcagcgtcagccctttatccgccacgtctaccgtata

SEQ ID NO: 23 - DNA, 54 bp, Artificial Sequence
  oligo-199
cggctgaattcaaaggcaccttcgaagaggcgaccgcgaaggcctacgcgtatg

SEQ ID NO: 24 - DNA, 30 bp, Artificial Sequence
  oligo-201
cttggcgaggaggtctgcatacgcgtaggc

SEQ ID NO: 25 - DNA, 63 bp, Artificial Sequence
  oligo-200
ctcctcgccaaggagaacggggaatatacggccgatcttgaggatggcgggaatacgatcaac

SEQ ID NO: 26 - DNA, 32 bp, Artificial Sequence
  oligo-197
ggctcgcattagagacgccggaagaaccgaag

SEQ ID NO: 27 - DNA, 34 bp, Artificial Sequence
  oligo-198
ttgaattcagccgtctggatcttcccatccgcaa

SEQ ID NO: 28 - DNA, 30 bp, Artificial Sequence
  oligo-202
cttggcgaggaggtttgcatacgcgtaggc

SEQ ID NO: 29 - DNA, 48 bp, Artificial Sequence
  oligo-203
aaagatcaggttaacgcggatcgtcacttcctcgcgcggttcttccgg

SEQ ID NO: 30 - DNA, 60 bp, Artificial Sequence
  oligo-204
gttaacctgatctttgcggatgggcgcacccagacggctgaattccgtggcaccttcgaa

SEQ ID NO: 31 - DNA, 30 bp, Artificial Sequence
  oligo-205
atattccccgttcacgcgggcgaggagatc

SEQ ID NO: 32 - DNA, 30 bp, Artificial Sequence
  oligo-206
gcagatctcctcgcccgcgtgaacggggaa

SEQ ID NO: 33 - DNA, 30 bp, Artificial Sequence
  oligo-207
aggcccccgcaaagcgaatgttgatcgtat

SEQ ID NO: 34 - DNA, 40 bp, Artificial Sequence
  oligo-210
acaggcgctagcatatggggccttagagacgccggaagaa

SEQ ID NO: 35 - DNA, 30 bp, Artificial Sequence
  oligo-211
tcttgctcggtaaggccccggcaaagcgaa

SEQ ID NO: 36 - protein, 322 aa, Artificial Sequence
  Amino acid sequence of PL-424
AQHDEAGLALETPEEPREEVTIRVNLIFADGRTQTAEFRGTFEEATAEAYRYADLLARVNGEYTADLEDGGYTINIRFAGALETPEEPREEVTIRVNLIFADGRTQTAEFRGTFEEATAEAYRYADLLARVNGEYTADLEDGGYTINIRFAGALETPEEPREEVTIRVNLIFADGRTQTAEFRGTFEEATAEAYRYADLLARVNGEYTADLEDGGYTINIRFAGALETPEEPREEVTIRVNLIFADGRTQTAEFRGTFEEATAEAYRYADLLARVNGEYTADLEDGGYTINIRFAGALPSKSKKILKEAKKLNKAQAPKKKK

SEQ ID NO: 37 - protein, 466 aa, Artificial Sequence
  Amino acid sequence of PL-624
AQHDEAGLALETPEEPREEVTIRVNLIFADGRTQTAEFRGTFEEATAEAYRYADLLARVNGEYTADLEDGGYTINIRFAGALETPEEPREEVTIRVNLIFADGRTQTAEFRGTFEEATAEAYRYADLLARVNGEYTADLEDGGYTINIRFAGALETPEEPREEVTIRVNLIFADGRTQTAEFRGTFEEATAEAYRYADLLARVNGEYTADLEDGGYTINIRFAGALETPEEPREEVTIRVNLIFADGRTQTAEFRGTFEEATAEAYRYADLLARVNGEYTADLEDGGYTINIRFAGALETPEEPREEVTIRVNLIFADGRTQTAEFRGTFEEATAEAYRYADLLARVNGEYTADLEDGGYTINIRFAGALETPEEPREEVTIRVNLIFADGRTQTAEFRGTFEEATAEAYRYADLLARVNGEYTADLEDGGYTINIRFAGALPSKSKKILKEAKKLNKAQAPKKKK

SEQ ID NO: 38 - DNA, 30 bp, Artificial Sequence
  oligo-334
gaattcagccgtctggatgcgcccatccgc

SEQ ID NO: 39 - DNA, 29 bp, Artificial Sequence
  oligo-335
ccagacggctgaattccgtggcaccttcg